European Patent Application EP 4 364 582 A1, published May 8, 2024. Title: The peptide compounds for flavor modulating. Applicant: CJ CheilJedang Corporation Technische Universitaet Muenchen. The sequence listing filed with the application follows.

SEQUENCE LISTING (26 sequences)

SEQ ID NO: 1 - protein, 7 aa, Artificial Sequence
  synthetic_longer peptide (1)
ALDPLPT

SEQ ID NO: 2 - protein, 4 aa, Artificial Sequence
  synthetic_longer peptide (2)
DGFP

SEQ ID NO: 3 - protein, 4 aa, Artificial Sequence
  synthetic_longer peptide (3)
DGML

SEQ ID NO: 4 - protein, 6 aa, Artificial Sequence
  synthetic_longer peptide (4)
DNEDTP

SEQ ID NO: 5 - protein, 3 aa, Artificial Sequence
  synthetic_longer peptide (5)
EEL

SEQ ID NO: 6 - protein, 3 aa, Artificial Sequence
  synthetic_longer peptide (6)
EEV

SEQ ID NO: 7 - protein, 3 aa, Artificial Sequence
  synthetic_longer peptide (7)
EEY

SEQ ID NO: 8 - protein, 7 aa, Artificial Sequence
  synthetic_longer peptide (8)
ESLPALP

SEQ ID NO: 9 - protein, 6 aa, Artificial Sequence
  synthetic_longer peptide (9)
EVGYGY

SEQ ID NO: 10 - protein, 4 aa, Artificial Sequence
  synthetic_longer peptide (10)
LDYY

SEQ ID NO: 11 - protein, 4 aa, Artificial Sequence
  synthetic_longer peptide (11)
LPPP

SEQ ID NO: 12 - protein, 6 aa, Artificial Sequence
  synthetic_longer peptide (12)
MTTFTW

SEQ ID NO: 13 - protein, 4 aa, Artificial Sequence
  synthetic_longer peptide (13)
PPPP

SEQ ID NO: 14 - protein, 5 aa, Artificial Sequence
  synthetic_longer peptide (14)
PPPPP

SEQ ID NO: 15 - protein, 4 aa, Artificial Sequence
  synthetic_longer peptide (15)
DAPL

SEQ ID NO: 16 - protein, 3 aa, Artificial Sequence
  synthetic_longer peptide (16)
DVL

SEQ ID NO: 17 - protein, 4 aa, Artificial Sequence
  synthetic_longer peptide (17)
GGPF

SEQ ID NO: 18 - protein, 4 aa, Artificial Sequence
  synthetic_longer peptide (18)
EVLK

SEQ ID NO: 19 - protein, 5 aa, Artificial Sequence
  synthetic_longer peptide (19)
FADSL

SEQ ID NO: 20 - protein, 3 aa, Artificial Sequence
  synthetic_longer peptide (20)
LAL

SEQ ID NO: 21 - protein, 3 aa, Artificial Sequence
  synthetic_longer peptide (21)
LLL

SEQ ID NO: 22 - protein, 3 aa, Artificial Sequence
  synthetic_longer peptide (22)
LLQ

SEQ ID NO: 23 - protein, 3 aa, Artificial Sequence
  synthetic_longer peptide (23)
LPL

SEQ ID NO: 24 - protein, 3 aa, Artificial Sequence
  synthetic_longer peptide (24)
PLL

SEQ ID NO: 25 - protein, 3 aa, Artificial Sequence
  synthetic_longer peptide (25)
TPL

SEQ ID NO: 26 - protein, 3 aa, Artificial Sequence
  synthetic_longer peptide (26)
VLL